European Patent Specification EP 3 571 217 B1, published June 21, 2023. Title: METHODS AND COMPOSITIONS FOR OBTAINING NATURAL COMPTENCE IN BACILLUS HOST CELLS. Applicant: Danisco US Inc. The sequence listing filed with the application follows.

SEQUENCE LISTING (22 sequences)

SEQ ID NO: 1 - DNA, 237 bp, Bacillus licheniformis
atgaaaaaccgacgatcagagagctggccgaatttcttcaaggggaaacgaaagagaaaaccgctccgattgcgccggcgccgtcccgtgcgaattatccggtgtcatccgcccaacggcgtatgtacatcctcaatcagctcgaagaagcaagcacgagctacaatgtgccggcggttctgcttctggaaggcgaattggataaggagcgtctggaagacgcgtttcgggccttga

SEQ ID NO: 2 - protein, 78 aa, Bacillus licheniformis
MKNRRSESWPNFFKGKRKRKPLRLRRRRPVRIIRCHPPNGVCTSSISSKKQARATMCRRFCFWKANWIRSVWKTRFGP

SEQ ID NO: 3 - DNA, 171 bp, Bacillus licheniformis
atggacaggcagaacaaagcgggattcagcctgccgaaaaacgcgactggtatcccgtttcatccgctcagcaacggatgtatgccctccatcatattgaaaagaacggaacgggctacaacatgccgtctgttctcatgctggaaggcgtacttgatacggatcgcttga

SEQ ID NO: 4 - protein, 56 aa, Bacillus licheniformis
MDRQNKAGFSLPKNATGIPFHPLSNGCMPSIILKRTERATTCRLFSCWKAYLIRIA

SEQ ID NO: 5 - DNA, 100 bp, Artificial Sequence
  promoter + 5'UTR
gcttttcttttggaagaaaatatagggaaaatggtacttgttaaaaattcggaatatttatacaatatcatatgtttcacattgaaaggggaggagaatc

SEQ ID NO: 6 - DNA, 44 bp, Artificial Sequence
  terminator sequence
tttttttaacttttttaccacctttgtgaaaaaagttaaaaaaa

SEQ ID NO: 7 - DNA, 25 bp, Artificial Sequence
  RBS
aacgaaagcaaggaggagcagacgt

SEQ ID NO: 8 - DNA, 20 bp, Artificial Sequence
  primer
aagctgctgtcccttcaaga

SEQ ID NO: 9 - DNA, 23 bp, Artificial Sequence
  primer
cttcgagctgattgaggatgtac

SEQ ID NO: 10 - DNA, 21 bp, Artificial Sequence
  primer
catgagaacagacggcatgtt

SEQ ID NO: 11 - DNA, 20 bp, Artificial Sequence
  primer
aagctgctgtcccttcaaga

SEQ ID NO: 12 - DNA, 20 bp, Artificial Sequence
  primer
cggcggtaacaggaacaatc

SEQ ID NO: 13 - DNA, 23 bp, Artificial Sequence
  primer
tctccaagataactacgaactgc

SEQ ID NO: 14 - DNA, 20 bp, Artificial Sequence
  primer
ccataaaccgccgatcatgg

SEQ ID NO: 15 - DNA, 19 bp, Artificial Sequence
  primer
cgtacggagattggggcat

SEQ ID NO: 16 - DNA, 18 bp, Artificial Sequence
  primer
actcgtgaacatgcgcat

SEQ ID NO: 17 - protein, 192 aa, Bacillus licheniformis
MSTEDMTKDTYEVNSSTMAVLPLGEGEKPASKILETDRTFRVNMKPFQIIERSCRYFGSSYAGRKAGTYEVIKVSHKPPIMVDHSNNIFLFPTFSSTRPQCGWLSHAHVHEFCAAKYDNTFVTFVNGETLELPVSISSFENQVYRTAWLRTKFIDRIEGNPMQKKQEFMLYPKEDRNQLIYEFILRELKKRY

SEQ ID NO: 18 - protein, 192 aa, Bacillus licheniformis
MSTEDMTKDTYEVNSSTMAVLPLGEGEKSASKILETDRTFRVNMKPFQIIERSCRYFGSSYAGRKAGTYEVIKVSHKPPIMVDHSNNIFLFPTFSSTRPQCGWLSHAHVHEFCAAKYDNTFVTFVNGETLELPVSISSFENQVYRTAWLRTKFIDRIEGNPMQKKQEFMLYPKEDRNQLIYEFILRELKKRY

SEQ ID NO: 19 - DNA, 803 bp, Bacillus licheniformis
gccctcaggaagaacatttcagccgctttgcgcttcttgaaaacgaggtggaattttattttgagaaaaaacaagccggtcttgaacagtttgtaaaaataaaaaaagaatgggtaaaagatattttaaaagaccgatatcaggatatgaaaaagaatcgtcttcaggccaaacctgatcaggagcctgttccgcttccgaagcaagcgaaaattaatcccgatgaaaaagtgattgccctcacatttgatgacggtccgaatcccgctacaacgaataaaatattaaacgctttacagaagcatgaagggcatgcgaccttctttgtgcttggaagcagagcccaatattatcccgaaacgataaaacggatgctgaaggaaggaaacgaagtcggcaaccattcctgggaccatccgttattgacaaggctgtcaaacgaaaaagcgtatcaggagattaacgacacgcaagaaatgatcgaaaaaatcagcggacacctgcctgtacacttgcgtcctccatacggcgggatcaatgattccgtccgctcgctttccaatctgaaggtttcattgtgggatgttgatccggaagattggaagtacaaaaataagcaaaagattgtcaatcatgtcatgagccatgcgggagacggaaaaatcgtcttaatgcacgatatttatgcaacgtccgcagatgctgctgaagagattattaaaaagctgaaagcaaaaggctatcaattggtaactgtatctcagcttgaagaagtgaagaagcagagaggctattgaggtacc

SEQ ID NO: 20 - DNA, 683 bp, Bacillus licheniformis
actagtatggcaacgttatctgatgtagcaaagaaagcaaatgtgtcgaaaatgacggtatcgcgggtgatcaatcatcctgagactgtgacggatgaattgaaaaagcttgttcattccgcaatgaaggagctcaattatataccgaactatgcagcaagagcgctcgttcaaaacagaacacaggtcgtcaagctgctcatactggaagaaatggatacaacagaaccttattatatgaatctgttaacgggaatcagccgcgagctggaccgtcatcattatgctttgcagcttgtcacaaggaaatctctcaatatcggccagtgcgacggcattattgcgacggggttgagaaaagccgattttgaagggctcatcaaggtttttgaaaagcctgtcgttgtattcgggcaaaatgaaatgggctacgattttattgatgttaacaatgaaaaaggaacctatatggcaacacgtcacgtcattggtctgggcgtccgcaatgtcgtcttttttgggatcgatttggatgagccctttgaacgctcaagggaaaaaggctatcttcaggcgatggaaggcagtctgaaaaaagcagcgattttccggatggaaaacagttcaaaaaaaagtgaagcacgcgcgcgggaagtgcttgcatcctttgacgcacctgcagc

SEQ ID NO: 21 - DNA, 237 bp, Bacillus licheniformis
ttgaaaaaccgacgatcagagagctggccgaatttcttcaaggggaaacgaaagagaaaaccgctccgattgcgccggcgccgtcccgtgcgaattatccggtgtcatccgcccaacggcgtatgtacatcctcaatcagctcgaagaagcaagcacgagctacaatgtgccggcggttctgcttctggaaggcgaattggataaggagcgtctggaagacgcgtttcgggccttga

SEQ ID NO: 22 - DNA, 171 bp, Bacillus licheniformis
atggacaggcagaacaaagcgggattcagcctgccgaaaaacgcgactggtatcccgtttcatccgctcagcaacggatgtatgccctccatcatattgaaaagaacggaacgggctacaacatgccgtctgttctcatgctggaaggcgtacttgatacggatcgcttaa